European Patent Application EP 4 215 204 A1, published July 26, 2023. Title: HUMAN NEUTROPHIL GELATINASE-ASSOCIATED LIPOCALIN DERIVED FROM RECOMBINANT BACTERIA AND USES THEREOF. Applicant: Universitat Pompeu Fabra. The sequence listing filed with the application follows.

SEQUENCE LISTING (16 sequences)

SEQ ID NO: 1 - protein, 178 aa, Artificial Sequence
  NGAL amino acid sequence without signalling peptide
QDSTSDLIPAPPLSKVPLQQNFQDNQFQGKWYVVGLAGNAILREDKDPQKMYATIYELKEDKSYNVTSVLFRKKKCDYWIRTFVPGCQPGEFTLGNIKSYPGLTSYLVRVVSTNYNQHAMVFFKKVSQNREYFKITLYGRTKELTSELKENFIRFSKSLGLPENHIVFPVPIDQCIDG

SEQ ID NO: 2 - DNA, 534 bp, Artificial Sequence
  NGAL nucleotide sequence without signalling peptide
caggactccacctccgacctcatcccggccccgccgctctccaaggtcccgctccagcagaacttccaggacaaccagttccagggcaagtggtacgtcgtcggcctcgccggcaacgccatcctccgcgaggacaaggacccgcagaagatgtacgccaccatctacgagctcaaggaggacaagtcctacaacgtcacctccgtcctcttccgcaagaagaagtgcgactactggatccgcaccttcgtcccgggctgccagccgggcgagttcaccctcggcaacatcaagtcctacccgggcctcacctcctacctcgtccgcgtcgtctccaccaactacaaccagcacgccatggtcttcttcaagaaggtctcccagaaccgcgagtacttcaagatcaccctctacggccgcaccaaggagctcacctccgagctcaaggagaacttcatccgcttctccaagtccctcggcctcccggagaaccacatcgtcttcccggtcccgatcgaccagtgcatcgacggc

SEQ ID NO: 3 - DNA, 69 bp, Artificial Sequence
  PPA1939 secretion peptide nucleotide sequence: (roxP)
atgttcgtccaaatcgctgccagcctggcagccgcatcgtccattgcactcggcataccaggagctgcc

SEQ ID NO: 4 - DNA, 84 bp, Artificial Sequence
  PPA0687 secretion peptide nucleotide sequence: (Camp2)
atgaagaagacccatcttgtagctcccctccttgtcggcgcaatgctcgtaccagcggcgctgtcagctcccagtgctcatgct

SEQ ID NO: 5 - DNA, 84 bp, Artificial Sequence
  PPA1340 secretion peptide nucleotide sequence: (camp1)
atgaaggttaagttcttagcagcgccgctggttgttggtgccttgatggcgccggcagctttctctggagcgacagctcatgct

SEQ ID NO: 6 - protein, 23 aa, Artificial Sequence
  PPA1939 secretion peptide amino acid sequence: (roxP)
MFVQIAASLAAASSIALGIPGAA

SEQ ID NO: 7 - protein, 28 aa, Artificial Sequence
  PPA0687 secretion peptide amino acid sequence: (Camp2
MKKTHLVAPLLVGAMLVPAALSAPSAHA

SEQ ID NO: 8 - protein, 28 aa, Artificial Sequence
  PPA1340 secretion peptide amino acid sequence: (camp1)
MKVKFLAAPLVVGALMAPAAFSGATAHA

SEQ ID NO: 9 - protein, 201 aa, Artificial Sequence
  NGAL amino acid sequence with signal peptide PPA1939
MFVQIAASLAAASSIALGIPGAAQDSTSDLIPAPPLSKVPLQQNFQDNQFQGKWYVVGLAGNAILREDKDPQKMYATIYELKEDKSYNVTSVLFRKKKCDYWIRTFVPGCQPGEFTLGNIKSYPGLTSYLVRVVSTNYNQHAMVFFKKVSQNREYFKITLYGRTKELTSELKENFIRFSKSLGLPENHIVFPVPIDQCIDG

SEQ ID NO: 10 - protein, 206 aa, Artificial Sequence
  NGAL amino acid sequence with signal peptide PPA0687
MKKTHLVAPLLVGAMLVPAALSAPSAHAQDSTSDLIPAPPLSKVPLQQNFQDNQFQGKWYVVGLAGNAILREDKDPQKMYATIYELKEDKSYNVTSVLFRKKKCDYWIRTFVPGCQPGEFTLGNIKSYPGLTSYLVRVVSTNYNQHAMVFFKKVSQNREYFKITLYGRTKELTSELKENFIRFSKSLGLPENHIVFPVPIDQCIDG

SEQ ID NO: 11 - protein, 206 aa, Artificial Sequence
  NGAL amino acid sequence with signal peptide PPA1340
MKVKFLAAPLVVGALMAPAAFSGATAHAQDSTSDLIPAPPLSKVPLQQNFQDNQFQGKWYVVGLAGNAILREDKDPQKMYATIYELKEDKSYNVTSVLFRKKKCDYWIRTFVPGCQPGEFTLGNIKSYPGLTSYLVRVVSTNYNQHAMVFFKKVSQNREYFKITLYGRTKELTSELKENFIRFSKSLGLPENHIVFPVPIDQCIDG

SEQ ID NO: 12 - DNA, 260 bp, Artificial Sequence
  PPA1340 promoter sequence: (Camp1)
taggttgactggaaaggggatatgacacccatcgtcctgggtctgacaggggtagacaatatagcttagaaatgtgtataagtaagatgtttctcgcaatgaaagacgatatgtcacgagttttctggtgctgtttcccgacacggaaccgttagtttgaatcaattttgaactgaggacaccaagttgaccccctggtgtgcaacgatgcttcttgcttgcagttgcgagcaattgttcccgatgaaaggaacccacaa

SEQ ID NO: 13 - DNA, 209 bp, Artificial Sequence
  PPA1939 promoter sequence: (RoxP)
acaccgacgatctgcacgggcgagtctaggggttatcggctacatgcgcgtcgccgcatcaggttcacgaaaccgaaaggcagacccaccccctaccgggcataccgttgccgccgacacttcgatgacactatgcagtgctacacttcaactgaaaatctatatgattttcgtcaattcccatacgtacgacacatcgggagatcgtc

SEQ ID NO: 14 - DNA, 200 bp, Artificial Sequence
  PPA0687 promoter sequence: (Camp2):
gcaacaagcctagacgggtctatgcaccgtcgtagccatacaccacacgggcccctgtcggaatgacgcacgcctgatcacagctccaacaaatgttggcggcgtacacgccgttcaccacaccgacccccatccaaaatatccgatacacttcgcttgcctcgaccggggcatccgcaaccaataaacggagaaccttt

SEQ ID NO: 15 - DNA, 5139 bp, Artificial Sequence
  pBR13 full plasmid sequence: suicide vector for targeting tdk locus (5139 bp)
ttgccgggaagctagagtaagtagttcgccagttaatagtttgcgcaacgttgttgccattgctacaggcatcgtggtgtcacgctcgtcgtttggtatggcttcattcagctccggttcccaacgatcaaggcgagttacatgatcccccatgttgtgcaaaaaagcggttagctccttcggtcctccgatcgttgtcagaagtaagttggccgcagtgttatcactcatggttatggcagcactgcataattctcttactgtcatgccatccgtaagatgcttttctgtgactggtgagtactcaaccaagtcattctgagaatagtgtatgcggcgaccgagttgctcttgcccggcgtcaatacgggataataccgcgccacatagcagaactttaaaagtgctcatcattggaaaacgttcttcggggcgaaaactctcaaggatcttaccgctgttgagatccagttcgatgtaacccactcgtgcacccaactgatcttcagcatcttttactttcaccagcgtttctgggtgagcaaaaacaggaaggcaaaatgccgcaaaaaagggaataagggcgacacggaaatgttgaatactcatactcttcctttttcaatattattgaagcatttatcagggttattgtctcatgagcggatacatatttgaatgtatttagaaaaataaacaaataggggttccgcgcacatttccccgaaaagtgccacctgatgcggtgtgaaataccgcacagatgcgtaaggagaaaataccgcatcaggaaattgtaagcgttaatattttgttaaaattcgcgttaaatttttgttaaatcagctcattttttaaccaataggccgaaatcggcaaaatcccttataaatcaaaagaatagaccgagatagggttgagtgttgttccagtttggaacaagagtccactattaaagaacgtggactccaacgtcaaagggcgaaaaaccgtctatcagggcgatggcccactacgtgaaccatcaccctaatcaagttttttggggtcgaggtgccgtaaagcactaaatcggaaccctaaagggagcccccgatttagagcttgacggggaaagccggcgaacgtggcgagaaaggaagggaagaaagcgaaaggagcgggcgctagggcgctggcaagtgtagcggtcacgctgcgcgtaaccaccacacccgccgcgcttaatgcgccgctacagggcgcgtccattcgccattcaggctgcgcaactgttgggaagggcgatcggtgcgggcctcttcgctattacgccagctggcgaaagggggatgtgctgcaaggcgattaagttgggtaacgccagggttttcccagtcacgacgttgtaaaacgacggccagtgaattgtaatacgactcactatagggcgaattgggcccgacgtcgcatgctcccggccgccatggcggccgcgggaattcgcccttccggccgccatggcgaaggatggcagtcggcagcatggagatcgcgcctcatgtgggttgacgagctcgttggtgctcttctcgatgagctcgatcctggaaccgccctggtcgtcactgctgatcacggcatggttgacatccccgacgaccaccgcgtcatggtggaggacgagggtggactgctcgctgacgttgccttgttggctggtgagcctcggttccgccacatttacactcgtcgtcccgatgaggtcgcgcaacgatggcgacgcgtactcggggatcgtgctcaggttgtcattggcgacgatgctgttgcggctgacctgtttggaccagttgacgtgtctacccgttcccgtttcggtgacgtactagcgattactcgtggtgattgggccatcatgagccgcgctacccccaaggaactcaccctcgtgggcatgcacggatcgctcactccgtgtgaaatgcggatcccattgctggcccagatctgtgaaggatgaggggtacctaggttgactggaaaggggatatgacacccatcgtcctgggtctgacaggggtagacaatatagcttagaaatgtgtataagtaagatgtttctcgcaatgaaagacgatatgtcacgagttttctggtgctgtttcccgacacggaaccgttagtttgaatcaattttgaactgaggacaccaagttgaccccctggtgtgcaacgatgcttcttgcttgcagttgcgagcaattgttcccgatgaaaggaacccacaaatggctagcatgttcgtccaaatcgctgccagcctggcagccgcatcgtccattgcactcggcataccaggagctgcccaggactccacctccgacctcatcccggccccgccgctctccaaggtcccgctccagcagaacttccaggacaaccagttccagggcaagtggtacgtcgtcggcctcgccggcaacgccatcctccgcgaggacaaggacccgcagaagatgtacgccaccatctacgagctcaaggaggacaagtcctacaacgtcacctccgtcctcttccgcaagaagaagtgcgactactggatccgcaccttcgtcccgggctgccagccgggcgagttcaccctcggcaacatcaagtcctacccgggcctcacctcctacctcgtccgcgtcgtctccaccaactacaaccagcacgccatggtcttcttcaagaaggtctcccagaaccgcgagtacttcaagatcaccctctacggccgcaccaaggagctcacctccgagctcaaggagaacttcatccgcttctccaagtccctcggcctcccggagaaccacatcgtcttcccggtcccgatcgaccagtgcatcgacggctctagaatcgaaggtcgtggcaagccgatcccgaacccgctcctcggcctcgactccacccgcaccggccaccaccatcaccaccattagtcgagcccggaggagaagagactgtgaacacgaacatgggcccacccctcaagaggaatgggcccatgccgtaaatgatttcgatgcaagtgtcaggacaacagcagggtaccatggctccaggtcctgacgagcgtggccccagggttcgcgtgcggtcaaggattttcccgcggtgggtggtatatcaggtatgcggggtggggccgccgaacatgatctcatcccaagaagggatcgacgcccgcttcgatttacgcggtttgcgcttcttgcgggggcggctaccctcctcgacgagggcgtcctgctggggagtctcatcggcagcttgagctgacgcttgtgagcgagaagtcgaagtcgaggtcttcttcgtcgatgtgcgtagcttcgacgccgcagtatcctgcgcggaggtgtcgtcatggggtggctgggcctcgcttttccccccagcctgatctggttgggatgtctcgatggcatgcggagccccggctggctggggagcctggggcgtagctggctcaggatcctgattcacctccggatgagacgcagcgtcaaggactggggtggcgagaccttcatagatgttgaccgagtcctcttgaaacccggcaagcacactagtgaattaagggcgaattcgcggccgcctgcaggtcgaccatatgggagagctcccaacgcgttggatgcatagcttgagtattctatagtgtcacctaaatagcttggcgtaatcatggtcatagctgtttcctgtgtgaaattgttatccgctcacaattccacacaacatacgagccggaagcataaagtgtaaagcctggggtgcctaatgagtgagctaactcacattaattgcgttgcgctcactgcccgctttccagtcgggaaacctgtcgtgccagctgcattaatgaatcggccaacgcgcggggagaggcggtttgcgtattgggcgctcttccgcttcctcgctcactgactcgctgcgctcggtcgttcggctgcggcgagcggtatcagctcactcaaaggcggtaatacggttatccacagaatcaggggataacgcaggaaagaacatgtgagcaaaaggccagcaaaaggccaggaaccgtaaaaaggccgcgttgctggcgtttttccataggctccgcccccctgacgagcatcacaaaaatcgacgctcaagtcagaggtggcgaaacccgacaggactataaagataccaggcgtttccccctggaagctccctcgtgcgctctcctgttccgaccctgccgcttaccggatacctgtccgcctttctcccttcgggaagcgtggcgctttctcatagctcacgctgtaggtatctcagttcggtgtaggtcgttcgctccaagctgggctgtgtgcacgaaccccccgttcagcccgaccgctgcgccttatccggtaactatcgtcttgagtccaacccggtaagacacgacttatcgccactggcagcagccactggtaacaggattagcagagcgaggtatgtaggcggtgctacagagttcttgaagtggtggcctaactacggctacactagaagaacagtatttggtatctgcgctctgctgaagccagttaccttcggaaaaagagttggtagctcttgatccggcaaacaaaccaccgctggtagcggtggtttttttgtttgcaagcagcagattacgcgcagaaaaaaaggatctcaagaagatcctttgatcttttctacggggtctgacgctcagtggaacgaaaactcacgttaagggattttggtcatgagattatcaaaaaggatcttcacctagatccttttaaattaaaaatgaagttttaaatcaatctaaagtatatatgagtaaacttggtctgacagttaccaatgcttaatcagtgaggcacctatctcagcgatctgtctatttcgttcatccatagttgcctgactccccgtcgtgtagataactacgatacgggagggcttaccatctggccccagtgctgcaatgataccgcgagacccacgctcaccggctccagatttatcagcaataaaccagccagccggaagggccgagcgcagaagtggtcctgcaactttatccgcctccatccagtctattaattg

SEQ ID NO: 16 - DNA, 9215 bp, Artificial Sequence
  pBR13 full plasmid sequence: replicative vector derivative of pBRESP36A (9215 bp)
gaattcaagcttgtcgacgttaacctgcaggcatgcggatccggtaccagcccgacccgagcacgcgccggcacgcctggtcgatgtcggaccggagttcgaggtacgcggcttgcaggtccaggaaggggacgtccatgcgagtgtccgttcgagtggcggcttgcgcccgatgctagtcgcggttgatcggcgatcgcaggtgcacgcggtcgatcttgacggctggcgagaggtgcggggaggatctgaccgacgcggtccacacgtggcaccgcgatgctgttgtgggctggacaatcgtgccggttggtaggatccagcggtgagcagttcggacgagcagccgcgcccgcgtcgccgcaaccaggatcggcagcaccccaaccagaaccggccggtgctgggccgtaccgagcgggaccgcaaccggcgccagttcgggcagaacttcctccgcgaccgcaagaccatcgcgcgcatcgccgagacagccgagctgcggcccgatctgccggtgctggaagccggccccgtcgaagggctgctcaccagggaactcgccgaccgcgcgcgtcaggtgacgtcgtacgagatcgacccccggctggcgaagtcgttgcgggagaagctttccggccacccgaacatcgaagtcgtcaacgccgacttcctcaccgccgaaccgccgcccgagccgttcgccttcgtcggcgcgatcccctacggcatcacctcggcgatcgtggactggtgcctggaggcgccgacgatcgagacggcgacgatggtcacgcagctggagttcgcccggaagcggaccggcgattacggccgctggagccgcctcacggtgatgacctggccgctgttcgagtgggagttcgtcgagaaggtcgaccgccggctgttcaagccggtgcccaaggtcgactcggcgatcatgcggctgcgcaggcgcgccgaaccgctgctggaaggcgcggcgctcgaacgctacgagtcgatggtcgagctgtgcttcaccggcgtcggcggcaacatccaggcgtcgcttctgcgcaagtacccgaggcgccgcgtcgaggcggcgttcgaccacgcgggggtcgggggcggcgccgtggtcgcctacgtccggccggagcagtggctccggctgttcgagcggctggatcagaagaacgaaccgaggggtgggcagccccagcggggcaggcgaaccggcggacgggaccacggggaccggcgaaccggcgggcaggatcgcggcgatcggcgaaccggcggccgcgaccacagggaccggcaagccagcggccacggcgatcgtcgcagcagcggacgcaatcgcgacgacggacgaaccggcgagcgcgagcagggggaccaaggcgggcggcgggggccgtccgggggtggacggaccggcggacgtccagggcgacgcggcggacccgggcagcggtagtccccggcacgcggaacgcggcaggccgtcgagcggcctgccccgttctgtcgagaggaatcagaggttgatgtcggcccggaggtcgatgtcgcgcgacgacgagccgatctccaccgctcgcttgccgcccccgagcttccagccgcccgcggcttcgtcccagtgctggagggccgctccgcgacgtgcacccggacgcgcttggtctcgcccggtgcgagttcgaccttctggtacctaggttgactggaaaggggatatgacacccatcgtcctgggtctgacaggggtagacaatatagcttagaaatgtgtataagtaagatgtttctcgcaatgaaagacgatatgtcacgagttttctggtgctgtttcccgacacggaaccgttagtttgaatcaattttgaactgaggacaccaagttgaccccctggtgtgcaacgatgcttcttgcttgcagttgcgagcaattgttcccgatgaaaggaacccacaaatggctagcatgttcgtccaaatcgctgccagcctggcagccgcatcgtccattgcactcggcataccaggagctgcccaggactccacctccgacctcatcccggccccgccgctctccaaggtcccgctccagcagaacttccaggacaaccagttccagggcaagtggtacgtcgtcggcctcgccggcaacgccatcctccgcgaggacaaggacccgcagaagatgtacgccaccatctacgagctcaaggaggacaagtcctacaacgtcacctccgtcctcttccgcaagaagaagtgcgactactggatccgcaccttcgtcccgggctgccagccgggcgagttcaccctcggcaacatcaagtcctacccgggcctcacctcctacctcgtccgcgtcgtctccaccaactacaaccagcacgccatggtcttcttcaagaaggtctcccagaaccgcgagtacttcaagatcaccctctacggccgcaccaaggagctcacctccgagctcaaggagaacttcatccgcttctccaagtccctcggcctcccggagaaccacatcgtcttcccggtcccgatcgaccagtgcatcgacggctctagaatcgaaggtcgtggcaagccgatcccgaacccgctcctcggcctcgactccacccgcaccggccaccaccatcaccaccattagtcgagcccggaggagaagagactgtgaacacgaacatgggcccacccctcaagaggaatgggcccatgccgtaaatgatttcgatgcaagtgtcaggacaacagcaggatcatccacgcaatgaaagcccgcacccaatacctcgaccagctctaaccaagaaaggaacctgatgagcgaccagctagacagcgaccgcaactacgacccgatgatcttcgacgtgatgcgcgagaccgcgaaccgcgtcgtcgccacgtacgttgcatgggaagatgaagccgctgatccccgcgaggctgcgcactggcaggccgagcgattccgcacccggcacgaggtgcgcgccgtcgaccctgacagccggcgagcagttcaggcgaagatcgcacagctgcgcgaggaactagccgcaatgcccgaacacgccccagccatcccttggagcaggtggcagcgtcaggggagtcgggggatgtttggcaggggatgtggaaagagagttcgctttgctcacatggctcaaccgggtaactaactgatatggggtcttcgtcgcccactttgaacacgccgaggaatggaccacgctgaacgtgactcgcatgcttcactgcatgtatggattcgttcgagacgttgttccctgagagctggctgccacgcaagccgctggcgtcagccgagaagtctggggcgtaccggcacgtgactcggcagagggcgctggagctgccttacatcgaagcgaacccgttggtcatgcagtccttggtcatcaccgatcgagatgcttcggatgctgactgggccgcagacctcgctgggctgccttcaccgtcctacgtgtccatgaaccgtgtcacgaccaccggacacatcgtctatgccttgaagaaccctgtgtgtctgaccgatgccgcgcggcgacggcctatcaacctgctcgcccgcgtcgagcagggcctatgcgacgttctcggcggcgatgcatcctacgggcaccggatcacaaagaacccgctcagcaccgcccatgcgaccctctggggccccgcagacgcgctctacgagctgcgcgccctcgcacacaccctcgacgagatccacgcactgccggaggcagggaacccgcgtcgcaacgtcacccgatcaacggtcggccgcaacgtcaccctgttcgacaccacccgcatgtgggcataccgggccgtccggcactcctggggcggcccggtcgccgaatgggagcacaccgtattcgagcacatccacctactgaacgagacgatcatcgccgacgaattcgccacaggccccctcggcttgaacgaacttaagcacttatctcgatccatttcccgatgggtctggcgcaacttcacccccgaaaccttccgcgcacgccagaaagcgatcagcctccgtggagcatccaaaggcggcaaagaaggcggccacaaaggcggcattgccagtggcgcatcacggcgcgcccatacccgtcaacagttcttggagggtctctcatgaccacacgtgaacgtctcccccgcaacggctacagcatcgccgctgctgcgaaaaagctcggtgtctccgagtccaccgtcaagcggtggacttccgagccacgcgaggagttcgtggcccgcgttgccgcacgccacgcgcggattcgtgagctccgctcggagggtcagagcatgcgtgcgattgctgccgaggtcggggtttccgtgggcaccgtgcactacgcgctgaacaagaatcgaactgacgcatgaccgtaacgccgcacgatgagcattttcttgatcgtgcaccgcttggcactacgttcgcgtgcggttgcacagtgcgcgccacgttcttatcctgcggccattgtggctacagccaatggggggcatcagcaacggacgttgaacccggtgggcaagtgttactcagggggacatgcccagtctgcggcgctcggattgacggtatggcagtcgtgcatgcggccccaccgtcaaactcattcaggtatcagtgagaaccctcatggcaccccctcgtgacacgttctcgttgcgatcagctgcggccaagcttgatcttcgggcagcgttgggtcctggccacgggtgcgcatgatcgtgctcctgtcgttgaggacccggctaggctggcggggttgccttactggttagcagaatgaatcaccgatacgcgagcgaacgtgaagcgactgctgctgcaaaacgtctgcgacctgagcaacaacatgaatggtcttcggtttccgtgtttcgtaaagtctggaaacgcggaagtcagcgccctgcaccattatgttccggatctgcatcgcaggatgctgctggctaccctgtggaacacctacatctgtattaacgaagcgctggcattgaccctgagtgatttttctctggtcccgccgcatccataccgccagttgtttaccctcacaacgttccagtaaccgggcatgttcatcatcagtaacccgtatcgtgagcatcctctctcgtttcatcggtatcattacccccatgaacagaaatcccccttacacggaggcatcagtgaccaaacaggaaaaaaccgcccttaacatggcccgctttatcagaagccagacattaacgcttctggagaaactcaacgagctggacgcggatgaacaggcagacatctgtgaatcgcttcacgaccacgctgatgagctttaccgcagctgcctcgcgcgtttcggtgatgacggtgaaaacctctgacacatgcagctcccggagacggtcacagcttgtctgtaagcggatgccgggagcagacaagcccgtcagggcgcgtcagcgggtgttggcgggtgtcggggcgcagccatgacccagtcacgtagcgatagcggagtgtatactggcttaactatgcggcatcagagcagattgtactgagagtgcaccatatgacccgaacatgtcgcgtgggtgcaaaatgagctcaacgaaacaccccgacaaatcctcggcggcgcaaccccacgtgaaatacttaacgaactattcaagcgtggcgcatccaccgcttgattccgccttgaaggcatgttagagtttggggcatgtcgagtcccgaatcagacaggtcaggggttgtcggtcacaccgccagccccttgaaccactagttacgacgcccacgatctgtgtgggcgtatgtctggcgtacccggggcgctggccgtggtgacaagaagaaccatttcttgatctcacacctcggagtactcgatgccttttgccctctacatgcttgccctggcggtcttcgtcatgggcacttcagaattcatgctcgcgggattgctccccgcgatcgcgaccgaacttgacgtctcggtcggcactgcgggcctgctgacctccgcattcgcagtcggtatggtcgtcggcgcgccagtgatggcggcattcgctcgccgttggccaccgcggctcacattgatcgtttgccttctcgtgttcgcgggaagccacgtcatcggagcgatgacaccagtgttctctctcctgctcatcacccgggtgctcagcgctctcgcaaacgcaggattcctcgccgtagcactgagcacggccactaccctcgtgccagcgaaccagaaggggcgtgcactgtcgatcctgctctccggcacgacgatcgcaaccgtcgtgggcgtccccgccggggcactgctcggcacagcgctgggctggcgaacgacgttctgggcgatcgccatcctctgtattcccgcggccgttggagtcattcgtggcgtcacgaacaatgttggtcggagcgagactagcgcgacctcaccaaggctccgtgtcgagctcagccagttggcgacgccgcggctcatcctggccatggcactcggagcgctgatcaacggagggacctttgcggcattcaccttcctggcacccatcgtgaccgagaccgcgggcttggccgaagcgtgggtgtccgtcgcgctggtgatgttcggcatcggatcgttccttggcgtcacgatcgcaggacgactatcagatcaacgacctggcctcgtgctcgcagtcggcggaccgctattgctgacaggctggatcgtgttggcagtggtcgcatctcatcccgttgcgcttatcgtcctcgtcctcgttcagggattcctgtcgttcggcgtcggcagtactctgatcacgcgtgtgctgtatgcagcatcgggtgcgccaacgatgggcggttcgtacgcaaccgcagcattgaatatcggagctgcagcggggcccgtgcttggtgcgctcgggctcgcgaccgggctggggctgctcgcgccggtttgggtcgcttcggtgctgacagcgatcgctctcgtcatcatgcttctcaccagacgcgcgcttacgaagaccgcggcggaggccaattgcatatgcggtgtgaaataccgcacagatgcgtaaggagaaaataccgcatcaggcgctcttccgcttcctcgctcactgactcgctgcgctcggtcgttcggctgcggcgagcggtatcagctcactcaaaggcggtaatacggttatccacagaatcaggggataacgcaggaaagaacatgtgagcaaaaggccagcaaaaggccaggaaccgtaaaaaggccgcgttgctggcgtttttccataggctccgcccccctgacgagcatcacaaaaatcgacgctcaagtcagaggtggcgaaacccgacaggactataaagataccaggcgtttccccctggaagctccctcgtgcgctctcctgttccgaccctgccgcttaccggatacctgtccgcctttctcccttcgggaagcgtggcgctttctcatagctcacgctgtaggtatctcagttcggtgtaggtcgttcgctccaagctgggctgtgtgcacgaaccccccgttcagcccgaccgctgcgccttatccggtaactatcgtcttgagtccaacccggtaagacacgacttatcgccactggcagcagccactggtaacaggattagcagagcgaggtatgtaggcggtgctacagagttcttgaagtggtggcctaactacggctacactagaagaacagtatttggtatctgcgctctgctgaagccagttaccttcggaaaaagagttggtagctcttgatccggcaaacaaaccaccgctggtagcggtggtttttttgtttgcaagcagcagattacgcgcagaaaaaaaggatctcaagaagatcctttgatcttttctacggggtctgacgctcagtggaacgaaaactcacgttaagggattttggtcatgagattatcaaaaaggatcttcacctagatccttttaaattaaaaatgaagttttaaatcaatctaaagtatatatgagtaaacttggtctgacagttaccaatgcttaatcagtgaggcacctatctcagcgatctgtctatttcgttcatccatagttgcctgactccccgtcgtgtagataactacgatacgggagggcttaccatctggccccagtgctgcaatgataccgcgagacccacgctcaccggctccagatttatcagcaataaaccagccagccggaagggccgagcgcagaagtggtcctgcaactttatccgcctccatccagtctattaattgttgccgggaagctagagtaagtagttcgccagttaatagtttgcgcaacgttgttgccattgctacaggcatcgtggtgtcacgctcgtcgtttggtatggcttcattcagctccggttcccaacgatcaaggcgagttacatgatcccccatgttgtgcaaaaaagcggttagctccttcggtcctccgatcgttgtcagaagtaagttggccgcagtgttatcactcatggttatggcagcactgcataattctcttactgtcatgccatccgtaagatgcttttctgtgactggtgagtactcaaccaagtcattctgagaatagtgtatgcggcgaccgagttgctcttgcccggcgtcaatacgggataataccgcgccacatagcagaactttaaaagtgctcatcattggaaaacgttcttcggggcgaaaactctcaaggatcttaccgctgttgagatccagttcgatgtaacccactcgtgcacccaactgatcttcagcatcttttactttcaccagcgtttctgggtgagcaaaaacaggaaggcaaaatgccgcaaaaaagggaataagggcgacacggaaatgttgaatactcatactcttcctttttcaatattattgaagcatttatcagggttattgtctcatgagcggatacatatttgaatgtatttagaaaaataaacaaataggggttccgcgcacatttccccgaaaagtgccacctgacgtctaagaaaccattattatcatgacattaacctataaaaataggcgtatcacgaggccctttcgtcttcaa